European Patent Application EP 4 464 333 A2, published November 20, 2024. Title: ANTI-DEATH RECEPTOR ANTIBODIES AND METHODS OF USE THEREOF. Applicant: Genmab B.V. Application EP PCT/EP2016/079517, filed December 1, 2016. The sequence listing filed with the application follows.

SEQUENCE LISTING (50 sequences)

SEQ ID NO: 1 - protein, 330 aa, Homo sapiens
ASTKGPSVFPLAPSSKSTSGGTAALGCLVKDYFPEPVTVSWNSGALTSGVHTFPAVLQSSGLYSLSSVVTVPSSSLGTQTYICNVNHKPSNTKVDKRVEPKSCDKTHTCPPCPAPELLGGPSVFLFPPKPKDTLMISRTPEVTCVVVDVSHEDPEVKFNWYVDGVEVHNAKTKPREEQYNSTYRVVSVLTVLHQDWLNGKEYKCKVSNKALPAPIEKTISKAKGQPREPQVYTLPPSREEMTKNQVSLTCLVKGFYPSDIAVEWESNGQPENNYKTTPPVLDSDGSFFLYSKLTVDKSRWQQGNVFSCSVMHEALHNHYTQKSLSLSPGK

SEQ ID NO: 2 - protein, 330 aa, Homo sapiens
ASTKGPSVFPLAPSSKSTSGGTAALGCLVKDYFPEPVTVSWNSGALTSGVHTFPAVLQSSGLYSLSSVVTVPSSSLGTQTYICNVNHKPSNTKVDKKVEPKSCDKTHTCPPCPAPELLGGPSVFLFPPKPKDTLMISRTPEVTCVVVDVSHEDPEVKFNWYVDGVEVHNAKTKPREEQYNSTYRVVSVLTVLHQDWLNGKEYKCKVSNKALPAPIEKTISKAKGQPREPQVYTLPPSREEMTKNQVSLTCLVKGFYPSDIAVEWESNGQPENNYKTTPPVLDSDGSFFLYSKLTVDKSRWQQGNVFSCSVMHEALHNHYTQKSLSLSPGK

SEQ ID NO: 3 - protein, 330 aa, Homo sapiens
ASTKGPSVFPLAPSSKSTSGGTAALGCLVKDYFPEPVTVSWNSGALTSGVHTFPAVLQSSGLYSLSSVVTVPSSSLGTQTYICNVNHKPSNTKVDKPVEPKSCDKTHTCPPCPAPELLGGPSVFLFPPKPKDTLMISRTPEVTCVVVDVSHEDPEVKFNWYVDGVEVHNAKTKPREEQYNSTYRVVSVLTVLHQDWLNGKEYKCKVSNKALPAPIEKTISKAKGQPREPQVYTLPPSRDELTKNQVSLTCLVKGFYPSDIAVEWESNGQPENNYKTTPPVLDSDGSFFLYSKLTVDKSRWQQGNVFSCSVMHEALHNHYTQKSLSLSPGK

SEQ ID NO: 4 - protein, 330 aa, Homo sapiens
ASTKGPSVFPLAPSSKSTSGGTAALGCLVKDYFPEPVTVSWNSGALTSGVHTFPAVLQSSGLYSLSSVVTVPSSSLGTQTYICNVNHKPSNTKVDKPVEPKSCDKTHTCPPCPAPELLGGPSVFLFPPKPKDTLMISRTPEVTCVVVDVSHEDPEVKFNWYVDGVEVHNAKTKPREEQYNSTYRVVSVLTVLHQDWLNGKEYKCKVSNKALPAPIEKTISKAKGQPREPQVYTLPPSREEMTKNQVSLTCLVKGFYPSDIAVEWESNGQPENNYKTTPPVLDSDGSFFLYSKLTVDKSRWQQGNVFSCSVMHEGLHNHYTQKSLSLSPGK

SEQ ID NO: 5 - protein, 330 aa, synthetic construct
ASTKGPSVFPLAPSSKSTSGGTAALGCLVKDYFPEPVTVSWNSGALTSGVHTFPAVLQSSGLYSLSSVVTVPSSSLGTQTYICNVNHKPSNTKVDKRVEPKSCDKTHTCPPCPAPELLGGPSVFLFPPKPKDTLMISRTPEVTCVVVDVSHEDPEVKFNWYVDGVEVHNAKTKPREEQYNSTYRVVSVLTVLHQDWLNGKEYKCKVSNKALPAPIEKTISKAKGQPREPQVYTLPPSREEMTKNQVSLTCLVKGFYPSDIAVEWESNGQPENNYKTTPPVLDSDGSFFLYSKLTVDKSRWQQGNVFSCSVMHGALHNHYTQKSLSLSPGK

SEQ ID NO: 6 - protein, 330 aa, synthetic construct
ASTKGPSVFPLAPSSKSTSGGTAALGCLVKDYFPEPVTVSWNSGALTSGVHTFPAVLQSSGLYSLSSVVTVPSSSLGTQTYICNVNHKPSNTKVDKRVEPKSCDKTHTCPPCPAPELLGGPSVFLFPPKPKDTLMISRTPEVTCVVVDVSHEDPEVKFNWYVDGVEVHNAKTKPREEQYNSTYRVVSVLTVLHQDWLNGKEYKCKVSNKALPAPIEKTISKAKGQPRKPQVYTLPPSREEMTKNQVSLTCLVKGFYPSDIAVEWESNGQPENNYKTTPPVLDSDGSFFLYSKLTVDKSRWQQGNVFSCSVMHEALHNHYTQKSLSLSPGK

SEQ ID NO: 7 - protein, 330 aa, synthetic construct
ASTKGPSVFPLAPSSKSTSGGTAALGCLVKDYFPEPVTVSWNSGALTSGVHTFPAVLQSSGLYSLSSVVTVPSSSLGTQTYICNVNHKPSNTKVDKRVEPKSCDKTHTCPPCPAPELLGGPSVFLFPPKPKDTLMISRTPEVTCVVVDVSHEDPEVKFNWYVDGVEVHNAKTKPREEQYNSTYRVVSVLTVLHQDWLNGKEYKCKVSNKALPAPIEKTISKAKGQPREPQVYTLPPSREEMTKNQVSLTCLVKGFYPSDIAVEWESNGQPENNYKTTPPVLDSDGSFFLYSKLTVDKSRWQQGNVFSCSVMHEALHNHYTQKYLSLSPGK

SEQ ID NO: 8 - protein, 330 aa, synthetic construct
ASTKGPSVFPLAPSSKSTSGGTAALGCLVKDYFPEPVTVSWNSGALTSGVHTFPAVLQSSGLYSLSSVVTVPSSSLGTQTYICNVNHKPSNTKVDKRVEPKSCDKTHTCPPCPAPELLGGPSVFLFPPKPKDTLMISRTPEVTCVVVDVSHEDPEVKFNWYVDGVEVHNAKTKPREEQYNSTYRVVSVLTVLHQDWLNGKEYKCKVSNKALPAPIEKTISKAKGQPREPQVYTLPPSREEMTKNQVSLTCLVKGFYPSDIAVEWESNGQPENNYKTTPPVLDSDGSFLLYSKLTVDKSRWQQGNVFSCSVMHEALHNHYTQKSLSLSPGK

SEQ ID NO: 9 - protein, 330 aa, synthetic construct
ASTKGPSVFPLAPSSKSTSGGTAALGCLVKDYFPEPVTVSWNSGALTSGVHTFPAVLQSSGLYSLSSVVTVPSSSLGTQTYICNVNHKPSNTKVDKRVEPKSCDKTHTCPPCPAPELLGGPSVFLFPPKPKDTLMISRTPEVTCVVVDVSHEDPEVKFNWYVDGVEVHNAKTKPREEQYNSTYRVVSVLTVLHQDWLNGKEYKCKVSNKALPAPIEKTISKAKGQPREPQVYTLPPSREEMTKNQVSLTCLVKGFYPSDIAVEWESNGQPENNYKTTPPVLDSDGSFFLYSRLTVDKSRWQQGNVFSCSVMHEALHNHYTQKSLSLSPGK

SEQ ID NO: 10 - protein, 330 aa, synthetic construct
ASTKGPSVFPLAPSSKSTSGGTAALGCLVKDYFPEPVTVSWNSGALTSGVHTFPAVLQSSGLYSLSSVVTVPSSSLGTQTYICNVNHKPSNTKVDKRVEPKSCDKTHTCPPCPAPELLGGPSVFLFPPKPKDTLMISRTPEVTCVVVDVSHEDPEVKFNWYVDGVEVHNAKTKPREEQYNSTYRVVSVLTVLHQDWLNGKEYKCKVSNKALPAPIEKTISKAKGQPREPQVYTLPPSREEMTKNQVSLTCLVKGFYPSDIAVEWESNGQPENNYKTTPPVLDSDGSFFLYSKLTVDKSRWQQGNVFSCSVMHEALHNHYTQESLSLSPGK

SEQ ID NO: 11 - protein, 330 aa, synthetic construct
ASTKGPSVFPLAPSSKSTSGGTAALGCLVKDYFPEPVTVSWNSGALTSGVHTFPAVLQSSGLYSLSSVVTVPSSSLGTQTYICNVNHKPSNTKVDKRVEPKSCDKTHTCPPCPAPELLGGPSVFLFPPKPKDTLMISRTPEVTCVVVDVSHEDPEVKFNWYVDGVEVHNAKTKPREEQYNSTYRVVSVLTVLHQDWLNGKEYKCKVSNKALPAPIEKTISKAKGQPREPQVYTLPPSREEMTKNQVSLTCLVKGFYPSDIAVEWESNGQPENNYKTTPPVLDSDGSFFLYSKLTVDKSRWQQGNVFSCSVMHEALHNHYTQKKLSLSPGK

SEQ ID NO: 12 - protein, 330 aa, synthetic construct
ASTKGPSVFPLAPSSKSTSGGTAALGCLVKDYFPEPVTVSWNSGALTSGVHTFPAVLQSSGLYSLSSVVTVPSSSLGTQTYICNVNHKPSNTKVDKRVEPKSCDKTHTCPPCPAPELLGGPSVFLFPPKPKDTLMISRTPEVTCVVVDVSHEDPEVKFNWYVDGVEVHNAKTKPREEQYNSTYRVVSVLTVLHQDWLNGKEYKCKVSNKALPAPIEKTISKAKGQPREPQVYTLPPSREEMTKNQVSLTCLVKGFYPSDIAVEWESNGQPENNYKTTPPVLDSDGSFFLYSKLTVDKSRWQQGNVFSCSVMHEALHNHITQKSLSLSPGK

SEQ ID NO: 13 - protein, 118 aa, synthetic construct
EVQLVQSGAEVKMPGASVKLSCRVSGDTFTAYFIHWVRQAPGQGLEWMGWFNPISGTAGSAEKFRGRVAMTRDTSISTAYMELNRLTFDDTAVYYCARQHRGNTFDPWGQGTLVTVSS

SEQ ID NO: 14 - protein, 111 aa, synthetic construct
QSALTQPASVSGSPGQSITISCTGTSSDIGAYKYVSWYQQHPGKAPKLVIYEVSNRPSGVSSRFSGSKSGQTASLTISGLQADDEADYYCNSYQGYNTWVFGGGTKVTVLG

SEQ ID NO: 15 - protein, 132 aa, synthetic construct
QLQLQESGPGLVKPSETLSLTCTVSGASISANSYYGVWVRQSPGKGLEWVGSIAYRGNSNSGSTYYNPSLKSRATVSVDTSKNQVSLRLTSVTAADTALYYCARRQLLDDGTGYQWAAFDVWGQGTMVTVSS

SEQ ID NO: 16 - protein, 110 aa, synthetic construct
QSVLTQPPSVSEAPRQTVTISCSGNSFNIGRYPVNWYQQLPGKAPKLLIYYNNLRFSGVSDRFSGSKSGTSASLAIRDLLSEDEADYYCSTWDDTLKGWVFGGGTKVTVL

SEQ ID NO: 17 - protein, 8 aa, synthetic construct
GFNIKDTF

SEQ ID NO: 18 - protein, 8 aa, synthetic construct
IDPANGNT

SEQ ID NO: 19 - protein, 11 aa, synthetic construct
VRGLYTYYFDY

SEQ ID NO: 20 - protein, 118 aa, synthetic construct
EVQLQQSGAEVVKPGASVKLSCKASGFNIKDTFIHWVKQAPGQGLEWIGRIDPANGNTKYDPKFQGKATITTDTSSNTAYMELSSLRSEDTAVYYCVRGLYTYYFDYWGQGTLVTVSS

SEQ ID NO: 21 - protein, 448 aa, synthetic construct
EVQLQQSGAEVVKPGASVKLSCKASGFNIKDTFIHWVKQAPGQGLEWIGRIDPANGNTKYDPKFQGKATITTDTSSNTAYMELSSLRSEDTAVYYCVRGLYTYYFDYWGQGTLVTVSSASTKGPSVFPLAPSSKSTSGGTAALGCLVKDYFPEPVTVSWNSGALTSGVHTFPAVLQSSGLYSLSSVVTVPSSSLGTQTYICNVNHKPSNTKVDKRVEPKSCDKTHTCPPCPAPELLGGPSVFLFPPKPKDTLMISRTPEVTCVVVDVSHEDPEVKFNWYVDGVEVHNAKTKPREEQYNSTYRVVSVLTVLHQDWLNGKEYKCKVSNKALPAPIEKTISKAKGQPREPQVYTLPPSREEMTKNQVSLTCLVKGFYPSDIAVEWESNGQPENNYKTTPPVLDSDGSFFLYSKLTVDKSRWQQGNVFSCSVMHEALHNHYTQKSLSLSPGK

SEQ ID NO: 22 - protein, 6 aa, synthetic construct
QSISNN

SEQ ID NO: 23 - protein, 9 aa, synthetic construct
QQGNSWPYT

SEQ ID NO: 24 - protein, 107 aa, synthetic construct
EIVMTQSPATLSVSPGERATLSCRASQSISNNLHWYQQKPGQAPRLLIKFASQSITGIPARFSGSGSGTEFTLTISSLQSEDFAVYYCQQGNSWPYTFGQGTKLEIK

SEQ ID NO: 25 - protein, 214 aa, synthetic construct
EIVMTQSPATLSVSPGERATLSCRASQSISNNLHWYQQKPGQAPRLLIKFASQSITGIPARFSGSGSGTEFTLTISSLQSEDFAVYYCQQGNSWPYTFGQGTKLEIKRTVAAPSVFIFPPSDEQLKSGTASVVCLLNNFYPREAKVQWKVDNALQSGNSQESVTEQDSKDSTYSLSSTLTLSKADYEKHKVYACEVTHQGLSSPVTKSFNRGEC

SEQ ID NO: 26 - protein, 8 aa, synthetic construct
IDPANTNT

SEQ ID NO: 27 - protein, 118 aa, synthetic construct
EVQLQQSGAEVVKPGASVKLSCKASGFNIKDTFIHWVKQAPGQGLEWIGRIDPANTNTKYDPKFQGKATITTDTSSNTAYMELSSLRSEDTAVYYCVRGLYTYYFDYWGQGTLVTVSS

SEQ ID NO: 28 - protein, 448 aa, synthetic construct
EVQLQQSGAEVVKPGASVKLSCKASGFNIKDTFIHWVKQAPGQGLEWIGRIDPANTNTKYDPKFQGKATITTDTSSNTAYMELSSLRSEDTAVYYCVRGLYTYYFDYWGQGTLVTVSSASTKGPSVFPLAPSSKSTSGGTAALGCLVKDYFPEPVTVSWNSGALTSGVHTFPAVLQSSGLYSLSSVVTVPSSSLGTQTYICNVNHKPSNTKVDKRVEPKSCDKTHTCPPCPAPELLGGPSVFLFPPKPKDTLMISRTPEVTCVVVDVSHEDPEVKFNWYVDGVEVHNAKTKPREEQYNSTYRVVSVLTVLHQDWLNGKEYKCKVSNKALPAPIEKTISKAKGQPREPQVYTLPPSREEMTKNQVSLTCLVKGFYPSDIAVEWESNGQPENNYKTTPPVLDSDGSFFLYSKLTVDKSRWQQGNVFSCSVMHEALHNHYTQKSLSLSPGK

SEQ ID NO: 29 - protein, 8 aa, synthetic construct
GFNIKDTH

SEQ ID NO: 30 - protein, 11 aa, synthetic construct
ARWGTNVYFAY

SEQ ID NO: 31 - protein, 118 aa, synthetic construct
QVQLVQSGAEVKKPGASVKVSCKASGFNIKDTHMHWVRQAPGQRLEWIGRIDPANGNTEYDQKFQGRVTITVDTSASTAYMELSSLRSEDTAVYYCARWGTNVYFAYWGQGTLVTVSS

SEQ ID NO: 32 - protein, 448 aa, synthetic construct
QVQLVQSGAEVKKPGASVKVSCKASGFNIKDTHMHWVRQAPGQRLEWIGRIDPANGNTEYDQKFQGRVTITVDTSASTAYMELSSLRSEDTAVYYCARWGTNVYFAYWGQGTLVTVSSASTKGPSVFPLAPSSKSTSGGTAALGCLVKDYFPEPVTVSWNSGALTSGVHTFPAVLQSSGLYSLSSVVTVPSSSLGTQTYICNVNHKPSNTKVDKRVEPKSCDKTHTCPPCPAPELLGGPSVFLFPPKPKDTLMISRTPEVTCVVVDVSHEDPEVKFNWYVDGVEVHNAKTKPREEQYNSTYRVVSVLTVLHQDWLNGKEYKCKVSNKALPAPIEKTISKAKGQPREPQVYTLPPSREEMTKNQVSLTCLVKGFYPSDIAVEWESNGQPENNYKTTPPVLDSDGSFFLYSKLTVDKSRWQQGNVFSCSVMHEALHNHYTQKSLSLSPGK

SEQ ID NO: 33 - protein, 5 aa, synthetic construct
SSVSY

SEQ ID NO: 34 - protein, 9 aa, synthetic construct
QQYHSYPPT

SEQ ID NO: 35 - protein, 106 aa, synthetic construct
DIQLTQSPSSLSASVGDRVTITCSASSSVSYMYWYQQKPGKAPKPWIYRTSNLASGVPSRFSGSGSGTDFTLTISSLQPEDFATYYCQQYHSYPPTFGGGTKVEIK

SEQ ID NO: 36 - protein, 213 aa, synthetic construct
DIQLTQSPSSLSASVGDRVTITCSASSSVSYMYWYQQKPGKAPKPWIYRTSNLASGVPSRFSGSGSGTDFTLTISSLQPEDFATYYCQQYHSYPPTFGGGTKVEIKRTVAAPSVFIFPPSDEQLKSGTASVVCLLNNFYPREAKVQWKVDNALQSGNSQESVTEQDSKDSTYSLSSTLTLSKADYEKHKVYACEVTHQGLSSPVTKSFNRGEC

SEQ ID NO: 37 - protein, 10 aa, synthetic construct
GGSISSGDYF

SEQ ID NO: 38 - protein, 7 aa, synthetic construct
IHNSGTT

SEQ ID NO: 39 - protein, 14 aa, synthetic construct
ARDRGGDYYYGMDV

SEQ ID NO: 40 - protein, 122 aa, synthetic construct
QVQLQESGPGLVKPSQTLSLTCTVSGGSISSGDYFWSWIRQLPGKGLECIGHIHNSGTTYYNPSLKSRVTISVDTSKKQFSLRLSSVTAADTAVYYCARDRGGDYYYGMDVWGQGTTVTVSS

SEQ ID NO: 41 - protein, 7 aa, synthetic construct
QGISRSY

SEQ ID NO: 42 - protein, 9 aa, synthetic construct
QQFGSSPWT

SEQ ID NO: 43 - protein, 108 aa, synthetic construct
EIVLTQSPGTLSLSPGERATLSCRASQGISRSYLAWYQQKPGQAPSLLIYGASSRATGIPDRFSGSGSGTDFTLTISRLEPEDFAVYYCQQFGSSPWTFGQGTKVEIK

SEQ ID NO: 44 - protein, 8 aa, synthetic construct
GFTFSSYV

SEQ ID NO: 45 - protein, 8 aa, synthetic construct
ISSGGSYT

SEQ ID NO: 46 - protein, 12 aa, synthetic construct
ARRGDSMITTDY

SEQ ID NO: 47 - protein, 449 aa, synthetic construct
EVMLVESGGGLVKPGGSLKLSCAASGFTFSSYVMSWVRQTPEKRLEWVATISSGGSYTYYPDSVKGRFTISRDNAKNTLYLQMSSLRSEDTAMYYCARRGDSMITTDYWGQGTTLTVSSASTKGPSVFPLAPSSKSTSGGTAALGCLVKDYFPEPVTVSWNSGALTSGVHTFPAVLQSSGLYSLSSVVTVPSSSLGTQTYICNVNHKPSNTKVDKRVEPKSCDKTHTCPPCPAPELLGGPSVFLFPPKPKDTLMISRTPEVTCVVVDVSHEDPEVKFNWYVDGVEVHNAKTKPREEQYNSTYRVVSVLTVLHQDWLNGKEYKCKVSNKALPAPIEKTISKAKGQPREPQVYTLPPSREEMTKNQVSLTCLVKGFYPSDIAVEWESNGQPENNYKTTPPVLDSDGSFFLYSKLTVDKSRWQQGNVFSCSVMHEALHNHYTQKSLSLSPGK

SEQ ID NO: 48 - protein, 6 aa, synthetic construct
QDVGTA

SEQ ID NO: 49 - protein, 8 aa, synthetic construct
QQYSSYRT

SEQ ID NO: 50 - protein, 213 aa, synthetic construct
DIVMTQSHKFMSTSVGDRVSITCKASQDVGTAVAWYQQKPGQSPKLLIYWASTRHTGVPDRFTGSGSGTDFTLTISNVQSEDLADYFCQQYSSYRTFGGGTKLEIKRTVAAPSVFIFPPSDEQLKSGTASVVCLLNNFYPREAKVQWKVDNALQSGNSQESVTEQDSKDSTYSLSSTLTLSKADYEKHKVYACEVTHQGLSSPVTKSFNRGEC